European Patent Specification EP 3 493 811 B1, published January 28, 2026. Title: SMALL MOLECULE THERAPEUTIC COMPOUNDS THAT REDUCE THE INCIDENCE OF INTRACEREBRAL HEMORRHAGE AND BRAIN MICROHEMORRHAGES. Applicant: St. Michael's Hospital. Application PCT/IB2017/001100. The sequence listing filed with the application follows.

SEQUENCE LISTING (17 sequences)

SEQ ID NO: 1 - DNA, 25 bp, Artificial Sequence
  Rap1bEx3
aaatgatgcagaacttgcctttctg

SEQ ID NO: 2 - DNA, 25 bp, Artificial Sequence
  cdh5exon2
tacaagaccgtctacctttccaatc

SEQ ID NO: 3 - DNA, 25 bp, Artificial Sequence
  ßPixexon6
gcgcatctctcttaccacattatag

SEQ ID NO: 4 - DNA, 25 bp, Artificial Sequence
  pak2aexon8
aatagagtacaacatacctcttggc

SEQ ID NO: 5 - DNA, 25 bp, Artificial Sequence
  Hmgcrb-splice
aactgcattcataaactcacccagt

SEQ ID NO: 6 - DNA, 25 bp, Artificial Sequence
  Pggtl-MO/ggtaseI splice
cacgcggtgtgtggactcacggtca

SEQ ID NO: 7 - DNA, 25 bp, Artificial Sequence
  Liss Std Control
cctcttacctcagttacaatttata

SEQ ID NO: 8 - DNA, 20 bp, Artificial Sequence
  VE-Cadherin Primer
acgatgtctccatcctgtct

SEQ ID NO: 9 - DNA, 20 bp, Artificial Sequence
  VE-Cadherin Primer
tagtgattcggttccctcat

SEQ ID NO: 10 - DNA, 20 bp, Artificial Sequence
  CCM1 Primer
tcacgctattcctgctctgt

SEQ ID NO: 11 - DNA, 20 bp, Artificial Sequence
  CCM1 Primer
actgcagatctgagccgtac

SEQ ID NO: 12 - DNA, 20 bp, Artificial Sequence
  CCM2 Primer
ggacagccagcattttgaga

SEQ ID NO: 13 - DNA, 20 bp, Artificial Sequence
  CCM2 Primer
gtctgaaatcatgcggtccc

SEQ ID NO: 14 - DNA, 19 bp, Artificial Sequence
  CCM3 Primer
catgattgacaggcccgag

SEQ ID NO: 15 - DNA, 20 bp, Artificial Sequence
  CCM3 Primer
tgattgtctgcaggaatcgg

SEQ ID NO: 16 - DNA, 20 bp, Artificial Sequence
  Integrin ß3 Primer
cacattcacagaacggaccc

SEQ ID NO: 17 - DNA, 20 bp, Artificial Sequence
  Integrin ß3 Primer
cacattcacagaacggaccc